European Patent Application EP 4 282 875 A2, published November 29, 2023. Title: REDUCED GLUTEN GRAINS AND COMPOSITIONS THEREOF. Applicant: Arcadia Biosciences, Inc. Application EP. The sequence listing filed with the application follows.

SEQUENCE LISTING (13 sequences)

SEQ ID NO: 1 - DNA, 2024 bp, Triticum aestivum
  source 1..2024: mol_type = genomic DNA
ctggcttgctcattttgcggtagtgtttaaacatcggctagccttacgggtataaaaaggtgggcaacttcaccctatcccatagcactagaccaaagaacacctatactccatactacccttcgttcacctggtgagcttcttcttcctttgatctatatcacttactatttctcccttgtccagcttcttcttcttcctcgtgcatgcgactttttctagataatatcccgcactatcgctcgccgcaagatgtgctagctagcgatcttcactttaatacctgttgtagatctaaccacgggctattccaaaaaatatttgtcttgtttgcgtgttcctgtgtacatgcacgtatctagatcttgattttgaagaattcataattaattcatgacctaccttgtttggtttgtgtaattttgatgttgtcgtatcaattttagcaaaccactcgtagctagaacaatagagggggcgatcgtatgtttctgttttgaaaaggggatatttccaggctctgcatcggttcatgcacacagccgttaccacattcaataggcactgatccatggatgcatgccagatttactagttttgtatacaaagttttacttttttgctttgatttatgaaaagttggatcagattttgcagttctcttttatccatgttggattcactactttgtacccaagattttatttattttgtcttggtttcttacctgcctggttagtaactaggagatcctgggattagactttcaaggaatcctaatactagtgagtatagggaaaggaagcttatttttaagctgcccaaaagaatgggcgcttagagttgtagttgattaattgaatctgttctgtggatttgagaatttcagacctgattctacatgacattttgagttaaccaatgattctacatgtctcactccttgggattaacaatttaactttatttaattcgatatgtgtgtacacatgtgttgcagatggaggaagtgtttccgtcaaactccaagagcaaggccggtcagatggcgggggaggcgacagcggcggcggagaagaagcctcggccgaagccagagcagaaggtggaatgccctcggtgcaagtctggcaacaccaagttctgctactacaacaactatagtatgtctcagccccgctacttctgcaaggcctgccgccgctactggacccatggtggctccctccgcaacgtccccatcggtggcggctgccgcaagcccaagcgcccggggacctccgacgcccacaagctcggcgtggcctcctcgtcagaacccacggttgtcatgccgccctcgacctgcacagggatgaactttgccaacgtcctcccaacatttatgtctgctggttttgagattccaagcagcctttccctgactgcctttgggtcatcgtcatcgtccaacacggcggcagtgatgtcccctggtgggacgacgtcatttctagacgtgttgagagggggcgcaggagggcttcttgatggcagcctcagtcagaacaatggctactactatggtgggcctgccactggatcaggcattgggatgctgatgacgccgccagtggcgtcatttggcattccaggtccgatgcagcaacatggtgatctcgtggttggtggaaatggaataggtgctgcaactgcttcaatatttcaggggggcactggcgaggaaggagatgatggtacggggggcgtgatggggctccaatggcagccacaggttggcaatggtggaggtgctggtgttgtatcaggaggcgtgcatcaccttgggactgggaacaatgtgacgatgggcaacaacaatatacacaacaacaacaataacaacagtgggggtgatgacaacaatggtgcgtcatcgagggattgctactggatcaacaatggaggatcgaacccatggcagagcctcctcaacaacagctccctgatgtaagtgcaataagaaaatgggaaatggaggtcat

SEQ ID NO: 2 - DNA, 990 bp, Triticum aestivum
  source 1..990: mol_type = unassigned DNA
atggaggaagtgtttccgtcaaactccaagagcaaggccggtcagatggcgggggaggcgacagcggcggcggagaagaagcctcggccgaagccagagcagaaggtggaatgccctcggtgcaagtctggcaacaccaagttctgctactacaacaactatagtatgtctcagccccgctacttctgcaaggcctgccgccgctactggacccatggtggctccctccgcaacgtccccatcggtggcggctgccgcaagcccaagcgcccggggacctccgacgcccacaagctcggcgtggcctcctcgtcagaacccacggttgtcatgccgccctcgacctgcacagggatgaactttgccaacgtcctcccaacatttatgtctgctggttttgagattccaagcagcctttccctgactgcctttgggtcatcgtcatcgtccaacacggcggcagtgatgtcccctggtgggacgacgtcatttctagacgtgttgagagggggcgcaggagggcttcttgatggcagcctcagtcagaacaatggctactactatggtgggcctgccactggatcaggcattgggatgctgatgacgccgccagtggcgtcatttggcattccaggtccgatgcagcaacatggtgatctcgtggttggtggaaatggaataggtgctgcaactgcttcaatatttcaggggggcactggcgaggaaggagatgatggtacggggggcgtgatggggctccaatggcagccacaggttggcaatggtggaggtgctggtgttgtatcaggaggcgtgcatcaccttgggactgggaacaatgtgacgatgggcaacaacaatatacacaacaacaacaataacaacagtgggggtgatgacaacaatggtgcgtcatcgagggattgctactggatcaacaatggaggatcgaacccatggcagagcctcctcaacaacagctccctgatg

SEQ ID NO: 3 - protein, 330 aa, Triticum aestivum
MEEVFPSNSKSKAGQMAGEATAAAEKKPRPKPEQKVECPRCKSGNTKFCYYNNYSMSQPRYFCKACRRYWTHGGSLRNVPIGGGCRKPKRPGTSDAHKLGVASSSEPTVVMPPSTCTGMNFANVLPTFMSAGFEIPSSLSLTAFGSSSSSNTAAVMSPGGTTSFLDVLRGGAGGLLDGSLSQNNGYYYGGPATGSGIGMLMTPPVASFGIPGPMQQHGDLVVGGNGIGAATASIFQGGTGEEGDDGTGGVMGLQWQPQVGNGGGAGVVSGGVHHLGTGNNVTMGNNNIHNNNNNNSGGDDNNGASSRDCYWINNGGSNPWQSLLNNSSLM

SEQ ID NO: 4 - DNA, 2028 bp, Triticum aestivum
  source 1..2028: mol_type = genomic DNA
ctggcttgctcattttgcggtagtgtttaaacattggctggaattacgggtataaaaaggagggcaacttcaccctatcccatagcactagaccaaacaactcctatactccatactacccttcattcacctggtgagcttcttctttctttgatttctatcacttactctttctccctcgtccagcttcttcttcttcctcgtgcatgtgacttttgctagataatctcccacattatcgctcaatgcaagccgtgctagctagctagcgatctagctagcgatcttcactttaatacccgttgtagatctaaccatgggctattccaaaacatatttctcttgtttgcgtgttcgtgtgtacatgcatgcatctagatcttgattttgaggaattcataagtaattcctgacctaccttgtttggtttgtttaattttgatgttgttgtctcaattttagcaaattgctcgtagctagaacaatagagggggcggccgtatgtttccgttttgaaaaggggatatttccaggctctgcatcggttgatgcacacagccgttaccacattcaataggcactgatccatggatgcatgctatatttacaagttttctatagaaattttttttatttatgaaaaattggatcggtatagttcttctttatccatgtcggattcactactttgtacccaagattttatttattttgtctcggtttcttacatgtctagttaggtaactaggagagcctgggattaggctttcaaggaatcctaatactagagactatggggagagacagcttattctttaagctgcgcaaaagaatgggcgcttagagttgtagttgataaattgaatctgttgtatggatttgagaatttgagacctgattatgcacttatcatgaaattttgagttaaccaatgattctacatgtctcactccttaggattaacaatttaacttaatttaattcgatatgtgtgtacacatgtgttgaagatggaggaagtgtttccgtcaaactccaagagcaaggctggtcagatggcgggggaggcgacagcggcggcggagaagaagcctcggccgaagccagagcagaaggtggaatgccctcggtgcaagtctggcaacaccaagttctgctactacaacaactatagtatgtctcagccccgctacttctgcaaggcctgccgccgctactggacccatggtgggtccctccgtaacgtccccatcggtggtggctgccgcaagcccaagcgctcggggacctccgacgcccacaagctcggcgtggcctcctcgtcggaacacacggctgtcatgcccccctcgacctgcacagggataaactttgccaatgtcctcccgacgtttatgtctgctggttttgagattccaagaagcctttccctgaccacctttgggtcatcgtcgtcgtccaacacgacggctgtcatgtcccctggtgggacgacgtcatttctagacgtgctgagagggggaacaggagggcttcttgatggcaacctcggtcagaacaatggctactactatggtgggtctagatcaggcattgggatgctgatgacgccgccagcggcgtcatttggcattccaggtccaatgcagcagcatggcgatctcatggttggtggaaatggaataggtgccgcaactgcttcaatatttcaggggggcactggtgaggaaggagatgacggcaaaggggccatgatggggctccaatggcagccacatgttggtaatggtggaggtggtggtgttgtatcaggaggcgtgcatcaccttgggactgggaacaatgtgacgatgggcaacaacaacataaacaacaataacaataatggcagccacagtgatgacaacactggtgggtcatcgagggattgctactggatcaataatggaggatcgaacccatggcaaagcctcctcaatagcagctccctgatgtaagtgcaagaagaaaatgcgaaatggagatcat

SEQ ID NO: 5 - DNA, 984 bp, Triticum aestivum
  source 1..984: mol_type = unassigned DNA
atggaggaagtgtttccgtcaaactccaagagcaaggctggtcagatggcgggggaggcgacagcggcggcggagaagaagcctcggccgaagccagagcagaaggtggaatgccctcggtgcaagtctggcaacaccaagttctgctactacaacaactatagtatgtctcagccccgctacttctgcaaggcctgccgccgctactggacccatggtgggtccctccgtaacgtccccatcggtggtggctgccgcaagcccaagcgctcggggacctccgacgcccacaagctcggcgtggcctcctcgtcggaacacacggctgtcatgcccccctcgacctgcacagggataaactttgccaatgtcctcccgacgtttatgtctgctggttttgagattccaagaagcctttccctgaccacctttgggtcatcgtcgtcgtccaacacgacggctgtcatgtcccctggtgggacgacgtcatttctagacgtgctgagagggggaacaggagggcttcttgatggcaacctcggtcagaacaatggctactactatggtgggtctagatcaggcattgggatgctgatgacgccgccagcggcgtcatttggcattccaggtccaatgcagcagcatggcgatctcatggttggtggaaatggaataggtgccgcaactgcttcaatatttcaggggggcactggtgaggaaggagatgacggcaaaggggccatgatggggctccaatggcagccacatgttggtaatggtggaggtggtggtgttgtatcaggaggcgtgcatcaccttgggactgggaacaatgtgacgatgggcaacaacaacataaacaacaataacaataatggcagccacagtgatgacaacactggtgggtcatcgagggattgctactggatcaataatggaggatcgaacccatggcaaagcctcctcaatagcagctccctgatg

SEQ ID NO: 6 - protein, 328 aa, Triticum aestivum
MEEVFPSNSKSKAGQMAGEATAAAEKKPRPKPEQKVECPRCKSGNTKFCYYNNYSMSQPRYFCKACRRYWTHGGSLRNVPIGGGCRKPKRSGTSDAHKLGVASSSEHTAVMPPSTCTGINFANVLPTFMSAGFEIPRSLSLTTFGSSSSSNTTAVMSPGGTTSFLDVLRGGTGGLLDGNLGQNNGYYYGGSRSGIGMLMTPPAASFGIPGPMQQHGDLMVGGNGIGAATASIFQGGTGEEGDDGKGAMMGLQWQPHVGNGGGGGVVSGGVHHLGTGNNVTMGNNNINNNNNNGSHSDDNTGGSSRDCYWINNGGSNPWQSLLNSSSLM

SEQ ID NO: 7 - DNA, 2081 bp, Triticum aestivum
  source 1..2081: mol_type = genomic DNA
ctggcttgctcattctgcggtagtgtttaaacatcagctagccttacgggtataaaaaggtgggcaacttcaccctatcccatagcactagaccaaacaacacctatactccatactacccttcattcacctggtgagattcttcttcctttgatctctatcacttactctttctcccttcttcttcttcttcttcttcttcttcttcttcttcttcttcttcttcttcttcttcttcttcctcgtgcatgctacttttgctacataatctcctgcagtatcgctcgccgcaagctgtgctagctagctagcgatcttcactttaagacccgttgtagatctagccacgggctattccaaaaaatatttctcttgtttgcgtgttcctgtgtacatgcatgtatttagatcttgatcttgaagaattcatactgaattcatgacctaccttgtttggtttgtgtaattttgatgttgttgtatcaattttagcaaaccgctcgtagctagaacaatagagggggcggccgtatgtttccatttcgaaaaggggatatttccaggctctgcatcggttcatgcacacagccgttaccacattcaataggcactaatccatggatgcatgccagatttactagttttgtttacaaagttttatttttttttgctttgatttacgaaaaattggatcggattttgcagttcttttttatccatgttggattcactactttgaacccaagattttatttattttgtctcggtttcttacacgcctggttaggtaactaggagatcctgggattaggctttcaaggaatcctaatactagagagtatggggagaggcaccttattttttaagttgcccaaaagaatgggcgcttagagttgtagctaattaattgaatctgttgtatggatctgagaatttgagacctgattatgcacttatcatgacattttgagtcaaccaatgattctacatgtctcactccttaggattaacaatttaacttaatttaattcgatatgtgtgtacacatgtgttgtagatggaggaagtgtttccgtcaaactccaagagcaaggcaggtcagatggcgggggaggcgatagcgggggcggagaagaagcctcggccaaagccagagcagaaggtggaatgccctcggtgcaagtctggcaacaccaagttctgctactacaacaactatagtatgtctcagccccgctacttctgcaaggcctgccgccgctactggacccatggtggctccctccgcaacgtccccatcggtggtggctgccgcaagcccaagcgctcggggacctccgacgcccacaagctcggcgtggcctcctcaccggaacccacgactgtcgtgcccccctcgacctgcacagggatgaactttgcgaacgtcctcccgacgtttatgtctgttggttttgagattccaagcagcctttccctaaccgcctttgggtcatcatcgtcgtccaacacggcggcgatgatgtcccctggtgggacgacgtcatttctagacgtgctaagagggggtgcaggagggcttcttgatggcagcctcagtcagaacaatggctactactatggtgggccagccattggatcaggcaatgggatgctgatgacgccgccagcggtgtcatttggcattccagttccgatgcagcagcatggtgatctcgtggttggtggaaatggaataggtgccgcaactgcttcaatatttcaaggggccactagcgaggaaggagatgacggcatggggggcgtgatggggctccaatggcaaccacaggttggcaatggtggaggtggtggtggtgtatcaggaggcgtgcatcaccttgggactgggaacaatgtgacgatgggcaacagcaacatacacaacaacaacaataacgacagcggcggtgatgacaacaatggtgggtcatcgagggattgctactggatcaacaatggaggatcaaacccatggcagagcctcctcaacagcagctccctgatgtaagtgcaagaagaaaatgggaaatggaggtcat

SEQ ID NO: 8 - DNA, 990 bp, Triticum aestivum
  source 1..990: mol_type = unassigned DNA
atggaggaagtgtttccgtcaaactccaagagcaaggcaggtcagatggcgggggaggcgatagcgggggcggagaagaagcctcggccaaagccagagcagaaggtggaatgccctcggtgcaagtctggcaacaccaagttctgctactacaacaactatagtatgtctcagccccgctacttctgcaaggcctgccgccgctactggacccatggtggctccctccgcaacgtccccatcggtggtggctgccgcaagcccaagcgctcggggacctccgacgcccacaagctcggcgtggcctcctcaccggaacccacgactgtcgtgcccccctcgacctgcacagggatgaactttgcgaacgtcctcccgacgtttatgtctgttggttttgagattccaagcagcctttccctaaccgcctttgggtcatcatcgtcgtccaacacggcggcgatgatgtcccctggtgggacgacgtcatttctagacgtgctaagagggggtgcaggagggcttcttgatggcagcctcagtcagaacaatggctactactatggtgggccagccattggatcaggcaatgggatgctgatgacgccgccagcggtgtcatttggcattccagttccgatgcagcagcatggtgatctcgtggttggtggaaatggaataggtgccgcaactgcttcaatatttcaaggggccactagcgaggaaggagatgacggcatggggggcgtgatggggctccaatggcaaccacaggttggcaatggtggaggtggtggtggtgtatcaggaggcgtgcatcaccttgggactgggaacaatgtgacgatgggcaacagcaacatacacaacaacaacaataacgacagcggcggtgatgacaacaatggtgggtcatcgagggattgctactggatcaacaatggaggatcaaacccatggcagagcctcctcaacagcagctccctgatg

SEQ ID NO: 9 - protein, 330 aa, Triticum aestivum
MEEVFPSNSKSKAGQMAGEAIAGAEKKPRPKPEQKVECPRCKSGNTKFCYYNNYSMSQPRYFCKACRRYWTHGGSLRNVPIGGGCRKPKRSGTSDAHKLGVASSPEPTTVVPPSTCTGMNFANVLPTFMSVGFEIPSSLSLTAFGSSSSSNTAAMMSPGGTTSFLDVLRGGAGGLLDGSLSQNNGYYYGGPAIGSGNGMLMTPPAVSFGIPVPMQQHGDLVVGGNGIGAATASIFQGATSEEGDDGMGGVMGLQWQPQVGNGGGGGGVSGGVHHLGTGNNVTMGNSNIHNNNNNDSGGDDNNGGSSRDCYWINNGGSNPWQSLLNSSSLM

SEQ ID NO: 10 - DNA, 189 bp, Triticum aestivum
  source 1..189: mol_type = unassigned DNA
aagccagagcagaaggtggaatgccctcggtgcaagtctggcaacaccaagttctgctactacaacaactatagtatgtctcagccccgctacttctgcaaggcctgccgccgctactggacccatggtggctccctccgcaacgtccccatcggtggtggctgccgcaagcccaagcgctcggggacc

SEQ ID NO: 11 - protein, 63 aa, Triticum aestivum
KPEQKVECPRCKSGNTKFCYYNNYSMSQPRYFCKACRRYWTHGGSLRNVPIGGGCRKPKRSGT

SEQ ID NO: 12 - DNA, 1011 bp, Hordeum vulgare
  source 1..1011: mol_type = unassigned DNA
atggaggaagtgttttcgtccaactccaagagcaaggccggtcagatggcgggagaggcggtggcggcggccgagaagaagtctcggccgaagccagagcagaaggtggagtgccctcggtgcaagtctggtaacaccaagttctgctactacaacaactacagcatgtcccagccgcgctacttctgcaaggcctgccgccgctactggacccatggtggctccctccgcaacgtccccatcggtggtggttgccgcaagcccaaacgcccggggacctctgacgcccacaagctcggcatggcctcctcatcggaacccacgggtgtcgtgcccccctcgaactgcacagggatgaactttgctaacgtcctcccgacgtttatgtctggtggctttgacattcaaagcagcctctccctgacaacttttgggtcatcatcctcatccaacccgacggggttgatgtcccccggtgggacgacttcatttctggatgtgctgagaggtggtgcaggagggcttcttgatggcagcctcggtccaaacaatggctactactatggtgggcatgccaatggatcaggcattgggatgttgatgactccgccaacggtatcgtttggcattccaagtccgatgcaacaacatggcggtctcgtggttggtggaaatggaataggtggcacaacttcttcaacatttcagggcaacgctggcgaggaaggagacgatggtacggggtccattatggggctccagtggcagccacatgttggtaatggtggcggtggtggtgttggattaggaggcgcgcatcatcttgggactgggaacaatgtgacgatgggcaacaacaacaataataacaaccagaacaacaataacggcggcggtgctggtgatgacgacgatggtgggtcatcgagggattgctactggatcaacaatggaggatcgaacccatggcagagcctcctcaacagcacctccctgatctcatacacacca

SEQ ID NO: 13 - protein, 337 aa, Hordeum vulgare
MEEVFSSNSKSKAGQMAGEAVAAAEKKSRPKPEQKVECPRCKSGNTKFCYYNNYSMSQPRYFCKACRRYWTHGGSLRNVPIGGGCRKPKRPGTSDAHKLGMASSSEPTGVVPPSNCTGMNFANVLPTFMSGGFDIQSSLSLTTFGSSSSSNPTGLMSPGGTTSFLDVLRGGAGGLLDGSLGPNNGYYYGGHANGSGIGMLMTPPTVSFGIPSPMQQHGGLVVGGNGIGGTTSSTFQGNAGEEGDDGTGSIMGLQWQPHVGNGGGGGVGLGGAHHLGTGNNVTMGNNNNNNNQNNNNGGGAGDDDDGGSSRDCYWINNGGSNPWQSLLNSTSLISYTP